European Patent Application EP 4 112 071 A9, published July 12, 2023. Title: NOVEL IMMUNIZATION AGENTS AND METHODS OF USE. Applicant: HSF Pharmaceuticals. The sequence listing filed with the application follows.

SEQUENCE LISTING (22 sequences)

SEQ ID NO: 1 - DNA, 21 bp, Homo sapiens
tcgacaactccgagtttcagc

SEQ ID NO: 2 - DNA, 39 bp, Homo sapiens
ctcctcgcggccgcatcgatccatagagcccaccgcatc

SEQ ID NO: 3 - DNA, 42 bp, herpes simplex virus 1
ctcctcaagcttctcgagcacacggagcgcggctgccgacac

SEQ ID NO: 4 - DNA, 35 bp, Herpes simplex virus 1
ctcctcggtaccccatggaggccagcagagccagc

SEQ ID NO: 5 - DNA, 42 bp, Herpes simplex virus 1
ctcctcgcggccgcactagttccgcgtgtccctttccgatgc

SEQ ID NO: 6 - DNA, 58 bp, Herpes simplex virus 1
ctcctcctcgagaagcttatgcatgagctcgacgtctcggcggtaatgagatacgagc

SEQ ID NO: 7 - DNA, 32 bp, Herpes simplex virus 1
ctcctcagaacccaggaccagggccacgttgg

SEQ ID NO: 8 - DNA, 33 bp, Herpes simplex virus 1
ctcctcatggagacaaagcccaagacggcaacc

SEQ ID NO: 9 - DNA, 36 bp, Herpes simplex virus 1
ctcctcggagaccggggttggggaatgaatccctcc

SEQ ID NO: 10 - DNA, 35 bp, Herpes simplex virus 1
ctcctcgcggggcgtgggaggggctggggcggacc

SEQ ID NO: 11 - DNA, 22 bp, Herpes simplex virus 1
agagggacatccaggactttgt

SEQ ID NO: 12 - DNA, 19 bp, Herpes simplex virus 1
caggcgcttgttggtgtac

SEQ ID NO: 13 - DNA, 16 bp, Herpes simplex virus 1
accgccgaactgagca

SEQ ID NO: 14 - DNA, 15 bp, Herpes simplex virus 1
cacgggccgcttcac

SEQ ID NO: 15 - DNA, 17 bp, Herpes simplex virus 1
gcgatagcgcgcgtaga

SEQ ID NO: 16 - DNA, 14 bp, Herpes simplex virus 1
ccgacgcgacctcc

SEQ ID NO: 17 - DNA, 17 bp, Herpes simplex virus 1
cctccacgcccaaaagc

SEQ ID NO: 18 - DNA, 22 bp, Herpes simplex virus 1
ggtggtgttgttcttgggtttg

SEQ ID NO: 19 - DNA, 15 bp, Herpes simplex virus 1
ccccacgtccacccc

SEQ ID NO: 20 - DNA, 25 bp, mus musculus
ctcaagaaatctaacccctgactca

SEQ ID NO: 21 - DNA, 16 bp, Mus musculus
gcgggacaggctgaga

SEQ ID NO: 22 - DNA, 15 bp, Mus musculus
ccccacacacacctc